European Patent Specification EP 3 486 312 B1, published November 22, 2023. Title: Leuconostoc mesenteroides CJLM627 producing decreased amounts of gas and methods for preparing kimchi using the same. Applicant: CJ Cheiljedang Corporation. The sequence listing filed with the application follows.

SEQUENCE LISTING (2 sequences)

SEQ ID NO: 1 - RNA, 962 nt, Unknown
  16s rRNA sequences of Leuconostoc mesenteroides CJLM627
ccactcggagtctccaggcggacacttaatgcgttagcttcggcactaagaggcggaaacctcctaacacctagtgttcatcgtttacggtgtggactaccagggtatctaatcctgtttgctacccacactttcgagcctcaacgtcagttgcagtccagtaagccgccttcgccactggtgttcttccatatatctacgcattccaccgctacacatggagttccacttacctctactgcactcaagttaaccagtttccaatgccattccggagttgagctccgggctttcacatcagacttaataaaccgtctgcgctcgctttacgcccaataaatccggataacgctcgggacatacgtattaccgcggctgctggcacgtatttagccgtccctttctggtatggtaccgtcaaactaaaatcatttcctattctagctgttcttcccatacaacagtgctttacgacccgaaagccttcatcacacacgcggcgttgctccatcaggctttcgcccattgtggaagattccctactgcagcctcccgtaggagtttgggccgtgtctcagtcccaatgtggccgatcagtctctcaactcggctatgcatcattgtcttggtaggcctttaccccaccaactaactaatgcaccgcggatccatctctaggtgacgccgaagcgccttttaactttgtgtcatgcgacactaagttttattcggtattagcatctgtttccaaatgttatccccagccttgaggcaggttgtccacgtgttactcacccgttcgccactcacttgaaaggtgcaagcacctttcgctgtgcgttcgacttgcatgtattaggcacgccgccagcgttcatctgacgaagaaaaacacatatatataaaaatgtacggaaaccaggagaacggaattttgggaacaaggtaaaagaaataaaagt

SEQ ID NO: 2 - RNA, 1507 nt, Unknown
  16s rRNA sequences of Leuconostoc mesenteroides subsp. dextranicum strain CCMMB1134
gctcaggatgaacgctggcggcgtgcctaatacatgcaagtcgaacgcacagcgaaaggtgcttgcacctttcaagtgagtggcgaacgggtgagtaacacgtggacaacctgcctcaaggctggggataacatttggaaacagatgctaataccgaataaaacttagtgtcgcatgacacaaagttaaaaggcgcttcggcgtcacctagagatggatccgcggtgcattagttagttggtggggtaaaggcctaccaagacaatgatgcatagccgagttgagagactgatcggccacattgggactgagacacggcccaaactcctacgggaggctgcagtagggaatcttccacaatgggcgaaagcctgatggagcaacgccgcgtgtgtgatgaaggctttcgggtcgtaaagcactgttgtatgggaagaacagctagaataggaaatgattttagtttgacggtaccataccagaaagggacggctaaatacgtgccagcagccgcggtaatacgtatgtcccgagcgttatccggatttattgggcgtaaagcgagcgcagacggtttattaagtctgatgtgaaagcccggagctcaactccggaatggcattggaaactggttaacttgagtgcagtagaggtaagtggaactccatgtgtagcggtggaatgcgtagatatatggaagaacaccagtggcgaaggcggcttactggactgcaactgacgttgaggctcgaaagtgtgggtagcaaacaggattagataccctggtagtccacaccgtaaacgatgaacactaggtgttaggaggtttccgcctcttagtgccgaagctaacgcattaagtgttccgcctggggagtacgaccgcaaggttgaaactcaaaggaattgacggggacccgcacaagcggtggagcatgtggtttaattcgaagcaacgcgaagaaccttaccaggtcttgacatcctttgaagcttttagagatagaagtgttctcttcggagacaaagtgacaggtggtgcatggtcgtcgtcagctcgtgtcgtgagatgttgggttaagtcccgcaacgagcgcaacccttattgttagttgccagcattcagatgggcactctagcgagactgccggtgacaaaccggaggaaggcggggacgacgtcagatcatcatgccccttatgacctgggctacacacgtgctacaatggcgtatacaacgagttgccaacccgcgagggtgagctaatctcttaaagtacgtctcagttcggattgtagtctgcaactcgactacatgaagtcggaatcgctagtaatcgcggatcagcacgccgcggtgaatacgttcccgggtcttgtacacaccgcccgtcacaccatgggagtttgtaatgcccaaagccggtggcctaaccttttaggaaggagccgtctaaggcaggacagatgactggggtgaagtcgtaacaaggtagccgtaggagaa